European Patent Specification EP 4 305 203 B1, published January 14, 2026. Title: High-Resolution Spatial Transciptome. Applicant: University of Washington. The sequence listing filed with the application follows.

SEQUENCE LISTING (18 sequences)

SEQ ID NO: 1 - DNA, 31 bp, Artificial Sequence
  sequencing primer site
gcggccgctaatacgactcactatagggatc

SEQ ID NO: 2 - DNA, 35 bp, Artificial Sequence
  sequencing primer site
cgaattccatcattgttcccgggttcctcattctc

SEQ ID NO: 3 - DNA, 368 bp, Artificial Sequence
  template structure
  misc_feature (63)..(84): n is a, c, g, or t
aatgatacggcgaccaccgagatctacactgcggccgctaatacgactcactatagggatctnnnnnnnnnnnnnnnnnnnnnnagagaatgaggaacccgggaacaatgatggaattttttttttttttttttttcgaaccaccgaggttgccggactagcgcaagtacttgtccattcctgaagaaatattatatttatacaacttacccatagaatcctatttactaggaaaggaaaagcctcctatttataaaaattggatagagctttctcaacaacagtggaatatcaatgatagaacaattgccgatttattagatggggtcttaataataccatcgatctcgtatgccgtcttctgcttg

SEQ ID NO: 4 - DNA, 29 bp, Artificial Sequence
  BA(+) probe
aatgatacggcgaccaccgagatctacac

SEQ ID NO: 5 - DNA, 24 bp, Artificial Sequence
  spatial index
  misc_feature (1)..(24): n is a, c, g, or t
nnnnnnnnnnnnnnnnnnnnnnnn

SEQ ID NO: 6 - DNA, 27 bp, Artificial Sequence
  sequencing priming site
ccaccgaggttgccggactagcgcaag

SEQ ID NO: 7 - DNA, 23 bp, Artificial Sequence
  BA(-) primer
tctcgtatgccgtcttctgcttg

SEQ ID NO: 8 - DNA, 368 bp, Artificial Sequence; identical to SEQ ID NO: 3
  template sequence
  misc_feature (63)..(84): n is a, c, g, or t

SEQ ID NO: 9 - DNA, 29 bp, Artificial Sequence
  polony bridge primer forward
aatgatacggcgaccaccgagatctacac

SEQ ID NO: 10 - DNA, 30 bp, Artificial Sequence
  spatial barcode forward sequencing primer
cggccgctaatacgactcactatagggatc

SEQ ID NO: 11 - DNA, 24 bp, Artificial Sequence
  spatial barcode
  misc_feature (1)..(6): n is a, c, g, or t
  misc_feature (7)..(9): nnn representsa spike sequence
  misc_feature (10)..(15): n is a, c, g, or t
  misc_feature (16)..(18): nnn representsa spike sequence
  misc_feature (19)..(24): n is a, c, g, or t
nnnnnnnnnnnnnnnnnnnnnnnn

SEQ ID NO: 12 - DNA, 31 bp, Artificial Sequence
  spatial barcode sequencing primer
gagaatgaggaacccgggaacaatgatggaa

SEQ ID NO: 13 - DNA, 20 bp, Artificial Sequence
  polyT primer for mRNA capture
tttttttttttttttttttt

SEQ ID NO: 14 - DNA, 27 bp, Artificial Sequence
  probe site
ccaccgaggttgccggactagcgcaag

SEQ ID NO: 15 - DNA, 24 bp, Artificial Sequence
  polony bridge primer reverse
atctcgtatgccgtcttctgcttg

SEQ ID NO: 16 - DNA, 29 bp, Artificial Sequence
  Primer BA(+)
aatgatacggcgaccaccgagatctacac

SEQ ID NO: 17 - DNA, 24 bp, Artificial Sequence
  Primer BA(-)
caagcagaagacggcatacgagat

SEQ ID NO: 18 - DNA, 34 bp, Artificial Sequence
  gene specific capturing primer
  misc_feature (1)..(8): n is a, c, g, or t
nnnnnnnntcgatcgattccatcattgttcccgg